European Patent Application EP 4 814 116 A1, published September 30, 2026. Title: Composition for editing nucleotide sequenc and method for editing nucleotide sequence using the same. Applicant: 国立大学法人広島大学. The sequence listing filed with the application follows.

SEQUENCE LISTING (232 sequences)

SEQ ID NO: 1 - DNA, 1491 bp, synthetic construct
  source 1..1491: mol_type = other DNA
  CDS 1..1491: protein_id = 2; translation = MVSKGEEVIKEFMRFKEHMEGSVNGHEFEIEGEGEGRPYEGTQTARLKVTKGGPLPFAWDILSPQIMYGSKAYVKHPADIPDYLKLSFPEGFKWERVMNFEDGGVVTVTQDSSLQDGEFIYKVKVRGTNFPSDGPVMQKKTMGWEASSERMYPEDGALKGEMKMRLRLKDGGHYDAEVKTTYMAKKPVQLPGAYKTDIKLDITSHNEDYTIVEQYERAEGRHSTGAGSREGRGSLLTCGDVEENPGPMESDESGLPAMEIECRITGTLNGVEFELVGGGEGTPKQGRMTNKMKSTKGALTFSPYLLSHVMGHGFYHFGTYPSGYENPFLHAINNGGYTNTRIEKYEDGGVLHVSFSYRYEAGRVIGDFKVVGTGFPEDSVIFTDKIIRSNATVEHLHPMGDNVLVGSFARTFSLRDGGYYSFVVDSHMHFKSAIHPSILQNGGPMFAFRRVEELHSNTELGIVEYQHAFKTPIAFARSRAQSSNSAVDGTAGPGST
atggtgagcaagggcgaggaggtcatcaaggagttcatgcgcttcaaggagcacatggagggctccgtgaacggccacgagttcgagatcgagggcgagggcgagggccgcccctacgagggcacccagaccgccaggctgaaggtgaccaagggtggccccctgcccttcgcctgggacatcctgtcccctcagatcatgtacggctccaaggcctacgtgaagcaccccgccgacatccccgactacttgaagctgtccttccccgagggcttcaagtgggagcgcgtgatgaacttcgaggacggcggcgtggtgaccgtgacccaggactcctccctgcaggacggcgagttcatctacaaggtgaaggtgcgcggcaccaacttcccctccgacggccccgtaatgcagaagaagaccatgggctgggaggcctcctccgagcggatgtaccccgaggacggcgccctgaagggcgagatgaagatgaggctgaggctgaaggacggcggccactacgacgccgaggtcaagaccacctacatggccaagaagcccgtgcagctgcccggcgcctacaagaccgacatcaagctggacatcacctcccacaacgaggactacaccatcgtggaacagtacgagcgcgccgagggccgccactccaccggcgccggatctcgcgagggcagaggaagtcttctaacatgcggtgacgtggaggagaatcccggccctatggagagcgacgagagcggcctgcccgccatggagatcgagtgccgcatcaccggcaccctgaacggcgtggagttcgagctggtgggcggcggagagggcacccccaagcagggccgcatgaccaacaagatgaagagcaccaaaggcgccctgaccttcagcccctacctgctgagccacgtgatgggccacggcttctaccacttcggcacctaccccagcggctacgagaaccccttcctgcacgccatcaacaacggcggctacaccaacacccgcatcgagaagtacgaggacggcggcgtgctgcacgtgagcttcagctaccgctacgaggccggccgcgtgatcggcgacttcaaggtggtgggcaccggcttccccgaggacagcgtgatcttcaccgacaagatcatccgcagcaacgccaccgtggagcacctgcaccccatgggcgataacgtgctggtgggcagcttcgcccgcaccttcagcctgcgcgacggcggctactacagcttcgtggtggacagccacatgcacttcaagagcgccatccaccccagcatcctgcagaacgggggccccatgttcgccttccgccgcgtggaggagctgcacagcaacaccgagctgggcatcgtggagtaccagcacgccttcaagacccccatcgccttcgccagatcccgcgctcagtcgtccaattctgccgtggacggcaccgccggacccggctccacctaa

SEQ ID NO: 2 - protein, 496 aa, synthetic construct
MVSKGEEVIKEFMRFKEHMEGSVNGHEFEIEGEGEGRPYEGTQTARLKVTKGGPLPFAWDILSPQIMYGSKAYVKHPADIPDYLKLSFPEGFKWERVMNFEDGGVVTVTQDSSLQDGEFIYKVKVRGTNFPSDGPVMQKKTMGWEASSERMYPEDGALKGEMKMRLRLKDGGHYDAEVKTTYMAKKPVQLPGAYKTDIKLDITSHNEDYTIVEQYERAEGRHSTGAGSREGRGSLLTCGDVEENPGPMESDESGLPAMEIECRITGTLNGVEFELVGGGEGTPKQGRMTNKMKSTKGALTFSPYLLSHVMGHGFYHFGTYPSGYENPFLHAINNGGYTNTRIEKYEDGGVLHVSFSYRYEAGRVIGDFKVVGTGFPEDSVIFTDKIIRSNATVEHLHPMGDNVLVGSFARTFSLRDGGYYSFVVDSHMHFKSAIHPSILQNGGPMFAFRRVEELHSNTELGIVEYQHAFKTPIAFARSRAQSSNSAVDGTAGPGST

SEQ ID NO: 3 - DNA, 1485 bp, synthetic construct
  source 1..1485: mol_type = other DNA
  CDS 1..1485: protein_id = 4; translation = MVSKGEEVIKEFMRFKEHMEGSVNGHEFEIEGEGEGRPYEGTQTARLKVTKGGPLPFAWDILSPQIMYGSKAYVKHPADIPDYLKLSFPEGFKWERVMNFEDGGVVTVTQDSSLQDGEFIYKVKVRGTNFPSDGPVMQKKTMGWEASSERMYPEDGALKGEMKMRLRLKDGGHYDAEVKTTYMAKKPVQLPGAYKTDIKLDITSHNEDYTIVEQYERAEGRHSTGAGSREGRGSLLTCGDVEENPGPMESDESGLMVSKGEELFTGVVPILVELDGDVNGHKFSVSGEGEGDATYGKLTLKFICTTGKLPVPWPTLVTTLTHGVQCFSRYPDHMKQHDFFKSAMPEGYVQERTIFFKDDGNYKTRAEVKFEGDTLVNRIELKGIDFKEDGNILGHKLEYNYNSHNVYIMADKQKNGIKVNFKIRHNIEDGSVQLADHYQQNTPIGDGPVLLPDNHYLSTQSKLSKDPNEKRDHMVLLEFVTAAGITLGMDELYK
atggtgagcaagggcgaggaggtcatcaaggagttcatgcgcttcaaggagcacatggagggctccgtgaacggccacgagttcgagatcgagggcgagggcgagggccgcccctacgagggcacccagaccgccaggctgaaggtgaccaagggtggccccctgcccttcgcctgggacatcctgtcccctcagatcatgtacggctccaaggcctacgtgaagcaccccgccgacatccccgactacttgaagctgtccttccccgagggcttcaagtgggagcgcgtgatgaacttcgaggacggcggcgtggtgaccgtgacccaggactcctccctgcaggacggcgagttcatctacaaggtgaaggtgcgcggcaccaacttcccctccgacggccccgtaatgcagaagaagaccatgggctgggaggcctcctccgagcggatgtaccccgaggacggcgccctgaagggcgagatgaagatgaggctgaggctgaaggacggcggccactacgacgccgaggtcaagaccacctacatggccaagaagcccgtgcagctgcccggcgcctacaagaccgacatcaagctggacatcacctcccacaacgaggactacaccatcgtggaacagtacgagcgcgccgagggccgccactccaccggcgccggatctcgcgagggcagaggaagtcttctaacatgcggtgacgtggaggagaatcccggccctatggagagcgacgagagcggcctgatggtgagcaagggcgaggagctgttcaccggggtggtgcccatcctggtcgagctggacggcgacgtaaacggccacaagttcagcgtgtccggcgagggcgagggcgatgccacctacggcaagctgaccctgaagttcatctgcaccaccggcaagctgcccgtgccctggcccaccctcgtgaccaccctgacccacggcgtgcagtgcttcagccgctaccccgaccacatgaagcagcacgacttcttcaagtccgccatgcccgaaggctacgtccaggagcgcaccatcttcttcaaggacgacggcaactacaagacccgcgccgaggtgaagttcgagggcgacaccctggtgaaccgcatcgagctgaagggcatcgacttcaaggaggacggcaacatcctggggcacaagctggagtacaactacaacagccacaacgtctatatcatggccgacaagcagaagaacggcatcaaggtgaacttcaagatccgccacaacatcgaggacggcagcgtgcagctcgccgaccactaccagcagaacacccccatcggcgacggccccgtgctgctgcccgacaaccactacctgagcacccagtccaagctgagcaaagaccccaacgagaagcgcgatcacatggtcctgctggagttcgtgaccgccgccgggatcactctcggcatggacgagctgtacaagtag

SEQ ID NO: 4 - protein, 494 aa, synthetic construct
MVSKGEEVIKEFMRFKEHMEGSVNGHEFEIEGEGEGRPYEGTQTARLKVTKGGPLPFAWDILSPQIMYGSKAYVKHPADIPDYLKLSFPEGFKWERVMNFEDGGVVTVTQDSSLQDGEFIYKVKVRGTNFPSDGPVMQKKTMGWEASSERMYPEDGALKGEMKMRLRLKDGGHYDAEVKTTYMAKKPVQLPGAYKTDIKLDITSHNEDYTIVEQYERAEGRHSTGAGSREGRGSLLTCGDVEENPGPMESDESGLMVSKGEELFTGVVPILVELDGDVNGHKFSVSGEGEGDATYGKLTLKFICTTGKLPVPWPTLVTTLTHGVQCFSRYPDHMKQHDFFKSAMPEGYVQERTIFFKDDGNYKTRAEVKFEGDTLVNRIELKGIDFKEDGNILGHKLEYNYNSHNVYIMADKQKNGIKVNFKIRHNIEDGSVQLADHYQQNTPIGDGPVLLPDNHYLSTQSKLSKDPNEKRDHMVLLEFVTAAGITLGMDELYK

SEQ ID NO: 5 - DNA, 79 bp, synthetic construct
  source 1..79: mol_type = other DNA
cgtagccgctggggtaggtgccgaagtggtagaagccgtagcccatcacgtggctcagcaggtaggggctgaaggtcag

SEQ ID NO: 6 - DNA, 35 bp, synthetic construct
  source 1..35: mol_type = other DNA
ctgaccttcagcccctacctgctgagccacgtgat

SEQ ID NO: 7 - DNA, 65 bp, synthetic construct
  source 1..65: mol_type = other DNA
ctcgtacttctcgatgcgggtgttggtgtagccgccgttgttgatggcgtgcaggaaggggttct

SEQ ID NO: 8 - DNA, 79 bp, synthetic construct
  source 1..79: mol_type = other DNA
tcatgtggtcggggtagcggctgaagcactgcacgccgtaggtcagggtggtcacgagggtgggccagggcacgggcag

SEQ ID NO: 9 - DNA, 35 bp, synthetic construct
  source 1..35: mol_type = other DNA
ctgcccgtgccctggcccaccctcgtgaccaccct

SEQ ID NO: 10 - DNA, 65 bp, synthetic construct
  source 1..65: mol_type = other DNA
gaagaagatggtgcgctcctggacgtagccttcgggcatggcggacttgaagaagtcgtgctgct

SEQ ID NO: 11 - DNA, 79 bp, synthetic construct; identical to SEQ ID NO: 5
  source 1..79: mol_type = other DNA
  modified_base 1^2: mod_base = OTHER; note = phosphorothioate bond
  modified_base 78^79: mod_base = OTHER; note = phosphorothioate bond

SEQ ID NO: 12 - DNA, 79 bp, synthetic construct; identical to SEQ ID NO: 5
  source 1..79: mol_type = other DNA
  modified_base 1^2: mod_base = OTHER; note = phosphorothioate bond

SEQ ID NO: 13 - DNA, 79 bp, synthetic construct; identical to SEQ ID NO: 5
  source 1..79: mol_type = other DNA
  modified_base 78^79: mod_base = OTHER; note = phosphorothioate bond

SEQ ID NO: 14 - DNA, 79 bp, synthetic construct; identical to SEQ ID NO: 5
  source 1..79: mol_type = other DNA
  modified_base 1^2: mod_base = OTHER; note = phosphorothioate bond
  modified_base 2^3: mod_base = OTHER; note = phosphorothioate bond
  modified_base 77^78: mod_base = OTHER; note = phosphorothioate bond
  modified_base 78^79: mod_base = OTHER; note = phosphorothioate bond

SEQ ID NO: 15 - DNA, 79 bp, synthetic construct; identical to SEQ ID NO: 5
  source 1..79: mol_type = other DNA
  modified_base 1^2: mod_base = OTHER; note = phosphorothioate bond
  modified_base 2^3: mod_base = OTHER; note = phosphorothioate bond

SEQ ID NO: 16 - DNA, 79 bp, synthetic construct; identical to SEQ ID NO: 5
  source 1..79: mol_type = other DNA
  modified_base 77^78: mod_base = OTHER; note = phosphorothioate bond
  modified_base 78^79: mod_base = OTHER; note = phosphorothioate bond

SEQ ID NO: 17 - DNA, 35 bp, synthetic construct; identical to SEQ ID NO: 6
  source 1..35: mol_type = other DNA
  modified_base 1^2: mod_base = OTHER; note = phosphorothioate bond
  modified_base 34^35: mod_base = OTHER; note = phosphorothioate bond

SEQ ID NO: 18 - DNA, 35 bp, synthetic construct; identical to SEQ ID NO: 6
  source 1..35: mol_type = other DNA
  modified_base 1^2: mod_base = OTHER; note = phosphorothioate bond

SEQ ID NO: 19 - DNA, 35 bp, synthetic construct; identical to SEQ ID NO: 6
  source 1..35: mol_type = other DNA
  modified_base 34^35: mod_base = OTHER; note = phosphorothioate bond

SEQ ID NO: 20 - DNA, 35 bp, synthetic construct; identical to SEQ ID NO: 6
  source 1..35: mol_type = other DNA
  modified_base 1^2: mod_base = OTHER; note = phosphorothioate bond
  modified_base 2^3: mod_base = OTHER; note = phosphorothioate bond
  modified_base 33^34: mod_base = OTHER; note = phosphorothioate bond
  modified_base 34^35: mod_base = OTHER; note = phosphorothioate bond

SEQ ID NO: 21 - DNA, 35 bp, synthetic construct; identical to SEQ ID NO: 6
  source 1..35: mol_type = other DNA
  modified_base 1^2: mod_base = OTHER; note = phosphorothioate bond
  modified_base 2^3: mod_base = OTHER; note = phosphorothioate bond

SEQ ID NO: 22 - DNA, 35 bp, synthetic construct; identical to SEQ ID NO: 6
  source 1..35: mol_type = other DNA
  modified_base 33^34: mod_base = OTHER; note = phosphorothioate bond
  modified_base 34^35: mod_base = OTHER; note = phosphorothioate bond

SEQ ID NO: 23 - DNA, 65 bp, synthetic construct; identical to SEQ ID NO: 7
  source 1..65: mol_type = other DNA
  modified_base 1^2: mod_base = OTHER; note = phosphorothioate bond
  modified_base 64^65: mod_base = OTHER; note = phosphorothioate bond

SEQ ID NO: 24 - DNA, 65 bp, synthetic construct; identical to SEQ ID NO: 7
  source 1..65: mol_type = other DNA
  modified_base 1^2: mod_base = OTHER; note = phosphorothioate bond

SEQ ID NO: 25 - DNA, 65 bp, synthetic construct; identical to SEQ ID NO: 7
  source 1..65: mol_type = other DNA
  modified_base 64^65: mod_base = OTHER; note = phosphorothioate bond

SEQ ID NO: 26 - DNA, 65 bp, synthetic construct; identical to SEQ ID NO: 7
  source 1..65: mol_type = other DNA
  modified_base 1^2: mod_base = OTHER; note = phosphorothioate bond
  modified_base 2^3: mod_base = OTHER; note = phosphorothioate bond
  modified_base 63^64: mod_base = OTHER; note = phosphorothioate bond
  modified_base 64^65: mod_base = OTHER; note = phosphorothioate bond

SEQ ID NO: 27 - DNA, 65 bp, synthetic construct; identical to SEQ ID NO: 7
  source 1..65: mol_type = other DNA
  modified_base 1^2: mod_base = OTHER; note = phosphorothioate bond
  modified_base 2^3: mod_base = OTHER; note = phosphorothioate bond

SEQ ID NO: 28 - DNA, 65 bp, synthetic construct; identical to SEQ ID NO: 7
  source 1..65: mol_type = other DNA
  modified_base 63^64: mod_base = OTHER; note = phosphorothioate bond
  modified_base 64^65: mod_base = OTHER; note = phosphorothioate bond

SEQ ID NO: 29 - DNA, 79 bp, synthetic construct; identical to SEQ ID NO: 5
  source 1..79: mol_type = other DNA
  modified_base 76^77: mod_base = OTHER; note = phosphorothioate bond
  modified_base 77^78: mod_base = OTHER; note = phosphorothioate bond
  modified_base 78^79: mod_base = OTHER; note = phosphorothioate bond

SEQ ID NO: 30 - DNA, 79 bp, synthetic construct; identical to SEQ ID NO: 5
  source 1..79: mol_type = other DNA
  modified_base 75^76: mod_base = OTHER; note = phosphorothioate bond
  modified_base 76^77: mod_base = OTHER; note = phosphorothioate bond
  modified_base 77^78: mod_base = OTHER; note = phosphorothioate bond
  modified_base 78^79: mod_base = OTHER; note = phosphorothioate bond

SEQ ID NO: 31 - DNA, 35 bp, synthetic construct; identical to SEQ ID NO: 6
  source 1..35: mol_type = other DNA
  modified_base 32^33: mod_base = OTHER; note = phosphorothioate bond
  modified_base 33^34: mod_base = OTHER; note = phosphorothioate bond
  modified_base 34^35: mod_base = OTHER; note = phosphorothioate bond

SEQ ID NO: 32 - DNA, 35 bp, synthetic construct; identical to SEQ ID NO: 6
  source 1..35: mol_type = other DNA
  modified_base 31^32: mod_base = OTHER; note = phosphorothioate bond
  modified_base 32^33: mod_base = OTHER; note = phosphorothioate bond
  modified_base 33^34: mod_base = OTHER; note = phosphorothioate bond
  modified_base 34^35: mod_base = OTHER; note = phosphorothioate bond

SEQ ID NO: 33 - DNA, 79 bp, synthetic construct; identical to SEQ ID NO: 5
  source 1..79: mol_type = other DNA
  modified_base 67^68: mod_base = OTHER; note = phosphorothioate bond
  modified_base 68^69: mod_base = OTHER; note = phosphorothioate bond

SEQ ID NO: 34 - DNA, 79 bp, synthetic construct; identical to SEQ ID NO: 5
  source 1..79: mol_type = other DNA
  modified_base 57^58: mod_base = OTHER; note = phosphorothioate bond
  modified_base 58^59: mod_base = OTHER; note = phosphorothioate bond

SEQ ID NO: 35 - DNA, 79 bp, synthetic construct; identical to SEQ ID NO: 5
  source 1..79: mol_type = other DNA
  modified_base 47^48: mod_base = OTHER; note = phosphorothioate bond
  modified_base 48^49: mod_base = OTHER; note = phosphorothioate bond

SEQ ID NO: 36 - DNA, 79 bp, synthetic construct; identical to SEQ ID NO: 5
  source 1..79: mol_type = other DNA
  modified_base 37^38: mod_base = OTHER; note = phosphorothioate bond
  modified_base 38^39: mod_base = OTHER; note = phosphorothioate bond

SEQ ID NO: 37 - DNA, 79 bp, synthetic construct; identical to SEQ ID NO: 5
  source 1..79: mol_type = other DNA
  modified_base 27^28: mod_base = OTHER; note = phosphorothioate bond
  modified_base 28^29: mod_base = OTHER; note = phosphorothioate bond

SEQ ID NO: 38 - DNA, 79 bp, synthetic construct; identical to SEQ ID NO: 5
  source 1..79: mol_type = other DNA
  modified_base 17^18: mod_base = OTHER; note = phosphorothioate bond
  modified_base 18^19: mod_base = OTHER; note = phosphorothioate bond

SEQ ID NO: 39 - DNA, 79 bp, synthetic construct; identical to SEQ ID NO: 5
  source 1..79: mol_type = other DNA
  modified_base 7^8: mod_base = OTHER; note = phosphorothioate bond
  modified_base 8^9: mod_base = OTHER; note = phosphorothioate bond

SEQ ID NO: 40 - DNA, 35 bp, synthetic construct; identical to SEQ ID NO: 6
  source 1..35: mol_type = other DNA
  modified_base 1^2: mod_base = OTHER; note = PCH3 modification
  modified_base 2^3: mod_base = OTHER; note = PCH3 modification

SEQ ID NO: 41 - DNA, 35 bp, synthetic construct; identical to SEQ ID NO: 6
  source 1..35: mol_type = other DNA
  modified_base 33^34: mod_base = OTHER; note = PCH3 modification
  modified_base 34^35: mod_base = OTHER; note = PCH3 modification

SEQ ID NO: 42 - DNA, 35 bp, synthetic construct; identical to SEQ ID NO: 6
  source 1..35: mol_type = other DNA
  modified_base 1^2: mod_base = OTHER; note = POCH2CH3 modification
  modified_base 2^3: mod_base = OTHER; note = POCH2CH3 modification

SEQ ID NO: 43 - DNA, 35 bp, synthetic construct; identical to SEQ ID NO: 6
  source 1..35: mol_type = other DNA
  modified_base 33^34: mod_base = OTHER; note = POCH2CH3 modification
  modified_base 34^35: mod_base = OTHER; note = POCH2CH3 modification

SEQ ID NO: 44 - DNA, 35 bp, synthetic construct; identical to SEQ ID NO: 6
  source 1..35: mol_type = other DNA
  modified_base 34^35: mod_base = OTHER; note = POCH2CH3 modification

SEQ ID NO: 45 - DNA, 35 bp, synthetic construct; identical to SEQ ID NO: 6
  source 1..35: mol_type = other DNA
  modified_base 33^34: mod_base = OTHER; note = POCH2CH3 modification
  modified_base 34^35: mod_base = OTHER; note = POCH2CH3 modification

SEQ ID NO: 46 - DNA, 79 bp, synthetic construct; identical to SEQ ID NO: 5
  source 1..79: mol_type = other DNA
  modified_base 40: mod_base = OTHER; note = 2'-O, 4'-C-methylene bridged nucleic acid

SEQ ID NO: 47 - DNA, 79 bp, synthetic construct; identical to SEQ ID NO: 5
  source 1..79: mol_type = other DNA
  modified_base 39..41: mod_base = OTHER; note = 2'-O, 4'-C-methylene bridged nucleic acid

SEQ ID NO: 48 - DNA, 79 bp, synthetic construct; identical to SEQ ID NO: 5
  source 1..79: mol_type = other DNA
  modified_base 39: mod_base = OTHER; note = 2'-O, 4'-C-methylene bridged nucleic acid
  modified_base 41: mod_base = OTHER; note = 2'-O, 4'-C-methylene bridged nucleic acid

SEQ ID NO: 49 - DNA, 79 bp, synthetic construct; identical to SEQ ID NO: 5
  source 1..79: mol_type = other DNA
  modified_base 37: mod_base = OTHER; note = 2'-O, 4'-C-methylene bridged nucleic acid
  modified_base 39: mod_base = OTHER; note = 2'-O, 4'-C-methylene bridged nucleic acid
  modified_base 41: mod_base = OTHER; note = 2'-O, 4'-C-methylene bridged nucleic acid
  modified_base 43: mod_base = OTHER; note = 2'-O, 4'-C-methylene bridged nucleic acid

SEQ ID NO: 50 - DNA, 79 bp, synthetic construct; identical to SEQ ID NO: 5
  source 1..79: mol_type = other DNA
  modified_base 35: mod_base = OTHER; note = 2'-O, 4'-C-methylene bridged nucleic acid
  modified_base 37: mod_base = OTHER; note = 2'-O, 4'-C-methylene bridged nucleic acid
  modified_base 39: mod_base = OTHER; note = 2'-O, 4'-C-methylene bridged nucleic acid
  modified_base 41: mod_base = OTHER; note = 2'-O, 4'-C-methylene bridged nucleic acid
  modified_base 43: mod_base = OTHER; note = 2'-O, 4'-C-methylene bridged nucleic acid
  modified_base 45: mod_base = OTHER; note = 2'-O, 4'-C-methylene bridged nucleic acid

SEQ ID NO: 51 - DNA, 79 bp, synthetic construct; identical to SEQ ID NO: 5
  source 1..79: mol_type = other DNA
  modified_base 38: mod_base = OTHER; note = 2'-O, 4'-C-methylene bridged nucleic acid
  modified_base 42: mod_base = OTHER; note = 2'-O, 4'-C-methylene bridged nucleic acid

SEQ ID NO: 52 - DNA, 79 bp, synthetic construct; identical to SEQ ID NO: 5
  source 1..79: mol_type = other DNA
  modified_base 38..39: mod_base = OTHER; note = 2'-O, 4'-C-methylene bridged nucleic acid
  modified_base 41..42: mod_base = OTHER; note = 2'-O, 4'-C-methylene bridged nucleic acid

SEQ ID NO: 53 - DNA, 79 bp, synthetic construct; identical to SEQ ID NO: 5
  source 1..79: mol_type = other DNA
  modified_base 37..38: mod_base = OTHER; note = 2'-O, 4'-C-methylene bridged nucleic acid
  modified_base 42..43: mod_base = OTHER; note = 2'-O, 4'-C-methylene bridged nucleic acid

SEQ ID NO: 54 - DNA, 79 bp, synthetic construct; identical to SEQ ID NO: 5
  source 1..79: mol_type = other DNA
  modified_base 37..39: mod_base = OTHER; note = 2'-O, 4'-C-methylene bridged nucleic acid
  modified_base 41..43: mod_base = OTHER; note = 2'-O, 4'-C-methylene bridged nucleic acid

SEQ ID NO: 55 - DNA, 79 bp, synthetic construct; identical to SEQ ID NO: 5
  source 1..79: mol_type = other DNA
  modified_base 33: mod_base = OTHER; note = 2'-O, 4'-C-methylene bridged nucleic acid
  modified_base 35: mod_base = OTHER; note = 2'-O, 4'-C-methylene bridged nucleic acid
  modified_base 37: mod_base = OTHER; note = 2'-O, 4'-C-methylene bridged nucleic acid
  modified_base 39: mod_base = OTHER; note = 2'-O, 4'-C-methylene bridged nucleic acid
  modified_base 41: mod_base = OTHER; note = 2'-O, 4'-C-methylene bridged nucleic acid
  modified_base 43: mod_base = OTHER; note = 2'-O, 4'-C-methylene bridged nucleic acid
  modified_base 45: mod_base = OTHER; note = 2'-O, 4'-C-methylene bridged nucleic acid
  modified_base 47: mod_base = OTHER; note = 2'-O, 4'-C-methylene bridged nucleic acid

SEQ ID NO: 56 - DNA, 79 bp, synthetic construct; identical to SEQ ID NO: 5
  source 1..79: mol_type = other DNA
  modified_base 31: mod_base = OTHER; note = 2'-O, 4'-C-methylene bridged nucleic acid
  modified_base 33: mod_base = OTHER; note = 2'-O, 4'-C-methylene bridged nucleic acid
  modified_base 35: mod_base = OTHER; note = 2'-O, 4'-C-methylene bridged nucleic acid
  modified_base 37: mod_base = OTHER; note = 2'-O, 4'-C-methylene bridged nucleic acid
  modified_base 39: mod_base = OTHER; note = 2'-O, 4'-C-methylene bridged nucleic acid
  modified_base 41: mod_base = OTHER; note = 2'-O, 4'-C-methylene bridged nucleic acid
  modified_base 43: mod_base = OTHER; note = 2'-O, 4'-C-methylene bridged nucleic acid
  modified_base 45: mod_base = OTHER; note = 2'-O, 4'-C-methylene bridged nucleic acid
  modified_base 47: mod_base = OTHER; note = 2'-O, 4'-C-methylene bridged nucleic acid
  modified_base 49: mod_base = OTHER; note = 2'-O, 4'-C-methylene bridged nucleic acid

SEQ ID NO: 57 - DNA, 79 bp, synthetic construct; identical to SEQ ID NO: 8
  source 1..79: mol_type = other DNA
  modified_base 38: mod_base = OTHER; note = 2'-O, 4'-C-methylene bridged nucleic acid
  modified_base 40: mod_base = OTHER; note = 2'-O, 4'-C-methylene bridged nucleic acid

SEQ ID NO: 58 - DNA, 35 bp, synthetic construct; identical to SEQ ID NO: 9
  source 1..35: mol_type = other DNA
  modified_base 34^35: mod_base = OTHER; note = POCH2CH3 modification

SEQ ID NO: 59 - DNA, 65 bp, synthetic construct; identical to SEQ ID NO: 10
  source 1..65: mol_type = other DNA

SEQ ID NO: 60 - DNA, 65 bp, synthetic construct
  source 1..65: mol_type = other DNA
cctcgtacttctcgatgcgggtgttggtgtagccgccgttgttgatggcgtgcaggaaggggttc

SEQ ID NO: 61 - DNA, 65 bp, synthetic construct
  source 1..65: mol_type = other DNA
tcctcgtacttctcgatgcgggtgttggtgtagccgccgttgttgatggcgtgcaggaaggggtt

SEQ ID NO: 62 - DNA, 65 bp, synthetic construct
  source 1..65: mol_type = other DNA
gtcctcgtacttctcgatgcgggtgttggtgtagccgccgttgttgatggcgtgcaggaaggggt

SEQ ID NO: 63 - DNA, 65 bp, synthetic construct
  source 1..65: mol_type = other DNA
gccgtcctcgtacttctcgatgcgggtgttggtgtagccgccgttgttgatggcgtgcaggaagg

SEQ ID NO: 64 - DNA, 65 bp, synthetic construct
  source 1..65: mol_type = other DNA
gccgccgtcctcgtacttctcgatgcgggtgttggtgtagccgccgttgttgatggcgtgcagga

SEQ ID NO: 65 - DNA, 65 bp, synthetic construct
  source 1..65: mol_type = other DNA
gtacttctcgatgcgggtgttggtgtagccgccgttgttgatggcgtgcaggaaggggttctcgt

SEQ ID NO: 66 - DNA, 65 bp, synthetic construct
  source 1..65: mol_type = other DNA
cttctcgatgcgggtgttggtgtagccgccgttgttgatggcgtgcaggaaggggttctcgtagc

SEQ ID NO: 67 - DNA, 65 bp, synthetic construct
  source 1..65: mol_type = other DNA
ctcgatgcgggtgttggtgtagccgccgttgttgatggcgtgcaggaaggggttctcgtagccgc

SEQ ID NO: 68 - DNA, 65 bp, synthetic construct
  source 1..65: mol_type = other DNA
gatgcgggtgttggtgtagccgccgttgttgatggcgtgcaggaaggggttctcgtagccgctgg

SEQ ID NO: 69 - DNA, 65 bp, synthetic construct
  source 1..65: mol_type = other DNA
gcgggtgttggtgtagccgccgttgttgatggcgtgcaggaaggggttctcgtagccgctggggt

SEQ ID NO: 70 - DNA, 65 bp, synthetic construct
  source 1..65: mol_type = other DNA
gtgttggtgtagccgccgttgttgatggcgtgcaggaaggggttctcgtagccgctggggtaggt

SEQ ID NO: 71 - DNA, 65 bp, synthetic construct
  source 1..65: mol_type = other DNA
agccgccgttgttgatggcgtgcaggaaggggttctcgtagccgctggggtaggtgccgaagtgg

SEQ ID NO: 72 - DNA, 65 bp, synthetic construct
  source 1..65: mol_type = other DNA
gttgatggcgtgcaggaaggggttctcgtagccgctggggtaggtgccgaagtggtagaagccgt

SEQ ID NO: 73 - DNA, 45 bp, synthetic construct
  source 1..45: mol_type = other DNA
caaaggcgccctgaccttcagcccctacctgctgagccacgtgat

SEQ ID NO: 74 - DNA, 55 bp, synthetic construct
  source 1..55: mol_type = other DNA
tgaagagcaccaaaggcgccctgaccttcagcccctacctgctgagccacgtgat

SEQ ID NO: 75 - DNA, 65 bp, synthetic construct
  source 1..65: mol_type = other DNA
accaacaagatgaagagcaccaaaggcgccctgaccttcagcccctacctgctgagccacgtgat

SEQ ID NO: 76 - DNA, 75 bp, synthetic construct
  source 1..75: mol_type = other DNA
gggccgcatgaccaacaagatgaagagcaccaaaggcgccctgaccttcagcccctacctgctgagccacgtgat

SEQ ID NO: 77 - DNA, 45 bp, synthetic construct
  source 1..45: mol_type = other DNA
ctgaccttcagcccctacctgctgagccacgtgatgggctacggc

SEQ ID NO: 78 - DNA, 55 bp, synthetic construct
  source 1..55: mol_type = other DNA
ctgaccttcagcccctacctgctgagccacgtgatgggctacggcttctaccact

SEQ ID NO: 79 - DNA, 65 bp, synthetic construct
  source 1..65: mol_type = other DNA
ctgaccttcagcccctacctgctgagccacgtgatgggctacggcttctaccacttcggcaccta

SEQ ID NO: 80 - DNA, 75 bp, synthetic construct
  source 1..75: mol_type = other DNA
ctgaccttcagcccctacctgctgagccacgtgatgggctacggcttctaccacttcggcacctaccccagcggc

SEQ ID NO: 81 - DNA, 79 bp, synthetic construct
  source 1..79: mol_type = other DNA
ctgaccttcagcccctacctgctgagccacgtgatgggctacggcttctaccacttcggcacctaccccagcggctacg

SEQ ID NO: 82 - DNA, 45 bp, synthetic construct
  source 1..45: mol_type = other DNA
ctgaccttcagcccctacctgctgagccacgtgatgggccacggc

SEQ ID NO: 83 - DNA, 55 bp, synthetic construct
  source 1..55: mol_type = other DNA
ctgaccttcagcccctacctgctgagccacgtgatgggccacggcttctaccact

SEQ ID NO: 84 - DNA, 65 bp, synthetic construct
  source 1..65: mol_type = other DNA
ctgaccttcagcccctacctgctgagccacgtgatgggccacggcttctaccacttcggcaccta

SEQ ID NO: 85 - DNA, 75 bp, synthetic construct
  source 1..75: mol_type = other DNA
ctgaccttcagcccctacctgctgagccacgtgatgggccacggcttctaccacttcggcacctaccccagcggc

SEQ ID NO: 86 - DNA, 79 bp, synthetic construct
  source 1..79: mol_type = other DNA
ctgaccttcagcccctacctgctgagccacgtgatgggccacggcttctaccacttcggcacctaccccagcggctacg

SEQ ID NO: 87 - DNA, 79 bp, synthetic construct
  source 1..79: mol_type = other DNA
agcccatcacgtggctcagcaggtaggggctgaaggtcagggcgcctttggtgctcttcatcttgttggtcatgcggcc

SEQ ID NO: 88 - DNA, 35 bp, synthetic construct
  source 1..35: mol_type = other DNA
ggccgcatgaccaacaagatgaagagcaccaaagg

SEQ ID NO: 89 - DNA, 65 bp, synthetic construct; identical to SEQ ID NO: 72
  source 1..65: mol_type = other DNA

SEQ ID NO: 90 - DNA, 79 bp, synthetic construct
  source 1..79: mol_type = other DNA
tagaagccgtagcccatcacgtggctcagcaggtaggggctgaaggtcagggcgcctttggtgctcttcatcttgttgg

SEQ ID NO: 91 - DNA, 35 bp, synthetic construct
  source 1..35: mol_type = other DNA
ccaacaagatgaagagcaccaaaggcgccctgacc

SEQ ID NO: 92 - DNA, 65 bp, synthetic construct; identical to SEQ ID NO: 71
  source 1..65: mol_type = other DNA

SEQ ID NO: 93 - DNA, 79 bp, synthetic construct
  source 1..79: mol_type = other DNA
gccgaagtggtagaagccgtagcccatcacgtggctcagcaggtaggggctgaaggtcagggcgcctttggtgctcttc

SEQ ID NO: 94 - DNA, 35 bp, synthetic construct
  source 1..35: mol_type = other DNA
gaagagcaccaaaggcgccctgaccttcagcccct

SEQ ID NO: 95 - DNA, 65 bp, synthetic construct; identical to SEQ ID NO: 70
  source 1..65: mol_type = other DNA

SEQ ID NO: 96 - DNA, 79 bp, synthetic construct
  source 1..79: mol_type = other DNA
tggggtaggtgccgaagtggtagaagccgtagcccatcacgtggctcagcaggtaggggctgaaggtcagggcgccttt

SEQ ID NO: 97 - DNA, 35 bp, synthetic construct
  source 1..35: mol_type = other DNA
aaaggcgccctgaccttcagcccctacctgctgag

SEQ ID NO: 98 - DNA, 65 bp, synthetic construct; identical to SEQ ID NO: 67
  source 1..65: mol_type = other DNA

SEQ ID NO: 99 - DNA, 79 bp, synthetic construct
  source 1..79: mol_type = other DNA
tcgtagccgctggggtaggtgccgaagtggtagaagccgtagcccatcacgtggctcagcaggtaggggctgaaggtca

SEQ ID NO: 100 - DNA, 35 bp, synthetic construct
  source 1..35: mol_type = other DNA
tgaccttcagcccctacctgctgagccacgtgatg

SEQ ID NO: 101 - DNA, 65 bp, synthetic construct; identical to SEQ ID NO: 60
  source 1..65: mol_type = other DNA

SEQ ID NO: 102 - DNA, 79 bp, synthetic construct
  source 1..79: mol_type = other DNA
ttctcgtagccgctggggtaggtgccgaagtggtagaagccgtagcccatcacgtggctcagcaggtaggggctgaagg

SEQ ID NO: 103 - DNA, 35 bp, synthetic construct
  source 1..35: mol_type = other DNA
ccttcagcccctacctgctgagccacgtgatgggc

SEQ ID NO: 104 - DNA, 65 bp, synthetic construct
  source 1..65: mol_type = other DNA
cgtcctcgtacttctcgatgcgggtgttggtgtagccgccgttgttgatggcgtgcaggaagggg

SEQ ID NO: 105 - DNA, 79 bp, synthetic construct
  source 1..79: mol_type = other DNA
gaaggggttctcgtagccgctggggtaggtgccgaagtggtagaagccgtagcccatcacgtggctcagcaggtagggg

SEQ ID NO: 106 - DNA, 35 bp, synthetic construct
  source 1..35: mol_type = other DNA
cccctacctgctgagccacgtgatgggctacggct

SEQ ID NO: 107 - DNA, 35 bp, synthetic construct
  source 1..35: mol_type = other DNA
cccctacctgctgagccacgtgatgggccacggct

SEQ ID NO: 108 - DNA, 65 bp, synthetic construct
  source 1..65: mol_type = other DNA
acgccgccgtcctcgtacttctcgatgcgggtgttggtgtagccgccgttgttgatggcgtgcag

SEQ ID NO: 109 - DNA, 79 bp, synthetic construct
  source 1..79: mol_type = other DNA
tggcgtgcaggaaggggttctcgtagccgctggggtaggtgccgaagtggtagaagccgtagcccatcacgtggctcag

SEQ ID NO: 110 - DNA, 35 bp, synthetic construct
  source 1..35: mol_type = other DNA
ctgagccacgtgatgggctacggcttctaccactt

SEQ ID NO: 111 - DNA, 35 bp, synthetic construct
  source 1..35: mol_type = other DNA
ctgagccacgtgatgggccacggcttctaccactt

SEQ ID NO: 112 - DNA, 65 bp, synthetic construct
  source 1..65: mol_type = other DNA
cacgtgcagcacgccgccgtcctcgtacttctcgatgcgggtgttggtgtagccgccgttgttga

SEQ ID NO: 113 - DNA, 79 bp, synthetic construct
  source 1..79: mol_type = other DNA
ccgttgttgatggcgtgcaggaaggggttctcgtagccgctggggtaggtgccgaagtggtagaagccgtagcccatca

SEQ ID NO: 114 - DNA, 35 bp, synthetic construct
  source 1..35: mol_type = other DNA
tgatgggctacggcttctaccacttcggcacctac

SEQ ID NO: 115 - DNA, 35 bp, synthetic construct
  source 1..35: mol_type = other DNA
tgatgggccacggcttctaccacttcggcacctac

SEQ ID NO: 116 - DNA, 65 bp, synthetic construct
  source 1..65: mol_type = other DNA
agctgaagctcacgtgcagcacgccgccgtcctcgtacttctcgatgcgggtgttggtgtagccg

SEQ ID NO: 117 - DNA, 79 bp, synthetic construct
  source 1..79: mol_type = other DNA
tgtagccgccgttgttgatggcgtgcaggaaggggttctcgtagccgctggggtaggtgccgaagtggtagaagccgta

SEQ ID NO: 118 - DNA, 35 bp, synthetic construct
  source 1..35: mol_type = other DNA
tacggcttctaccacttcggcacctaccccagcgg

SEQ ID NO: 119 - DNA, 35 bp, synthetic construct
  source 1..35: mol_type = other DNA
cacggcttctaccacttcggcacctaccccagcgg

SEQ ID NO: 120 - DNA, 65 bp, synthetic construct
  source 1..65: mol_type = other DNA
ggttgtgggcgtagctcttcatgctcctgccgccgcacgacgtgcactcgaagtcgatggcgatg

SEQ ID NO: 121 - DNA, 144 bp, synthetic construct
  source 1..144: mol_type = other DNA
ctcgtacttctcgatgcgggtgttggtgtagccgccgttgttgatggcgtgcaggaaggggttctcgtagccgctggggtaggtgccgaagtggtagaagccgtagcccatcacgtggctcagcaggtaggggctgaaggtcag

SEQ ID NO: 122 - DNA, 109 bp, synthetic construct
  source 1..109: mol_type = other DNA
cgttgttgatggcgtgcaggaaggggttctcgtagccgctggggtaggtgccgaagtggtagaagccgtagcccatcacgtggctcagcaggtaggggctgaaggtcag

SEQ ID NO: 123 - DNA, 35 bp, synthetic construct
  source 1..35: mol_type = other DNA
ctcgtacttctcgatgcgggtgttggtgtagccgc

SEQ ID NO: 124 - DNA, 65 bp, synthetic construct
  source 1..65: mol_type = other DNA
taggtgccgaagtggtagaagccgtagcccatcacgtggctcagcaggtaggggctgaaggtcag

SEQ ID NO: 125 - DNA, 79 bp, synthetic construct
  source 1..79: mol_type = other DNA
ctcgtacttctcgatgcgggtgttggtgtagccgccgttgttgatggcgtgcaggaaggggttctcgtagccgctgggg

SEQ ID NO: 126 - DNA, 35 bp, synthetic construct
  source 1..35: mol_type = other DNA
atcacgtggctcagcaggtaggggctgaaggtcag

SEQ ID NO: 127 - DNA, 109 bp, synthetic construct
  source 1..109: mol_type = other DNA
ctcgtacttctcgatgcgggtgttggtgtagccgccgttgttgatggcgtgcaggaaggggttctcgtagccgctggggtaggtgccgaagtggtagaagccgtagccc

SEQ ID NO: 128 - DNA, 79 bp, synthetic construct; identical to SEQ ID NO: 5
  source 1..79: mol_type = other DNA
  modified_base 1^2: mod_base = OTHER; note = phosphorothioate bond
  modified_base 39: mod_base = OTHER; note = 2'-O, 4'-C-methylene bridged nucleic acid
  modified_base 41: mod_base = OTHER; note = 2'-O, 4'-C-methylene bridged nucleic acid

SEQ ID NO: 129 - DNA, 65 bp, synthetic construct; identical to SEQ ID NO: 7
  source 1..65: mol_type = other DNA
  modified_base 1^2: mod_base = OTHER; note = phosphorothioate bond

SEQ ID NO: 130 - DNA, 79 bp, synthetic construct; identical to SEQ ID NO: 8
  source 1..79: mol_type = other DNA
  modified_base 39: mod_base = OTHER; note = 2'-O, 4'-C-methylene bridged nucleic acid
  modified_base 41: mod_base = OTHER; note = 2'-O, 4'-C-methylene bridged nucleic acid

SEQ ID NO: 131 - DNA, 79 bp, synthetic construct; identical to SEQ ID NO: 5
  source 1..79: mol_type = other DNA
  modified_base 39: mod_base = OTHER; note = 2'-O, 4'-C-ethylene bridged nucleic acid
  modified_base 41: mod_base = OTHER; note = 2'-O, 4'-C-ethylene bridged nucleic acid

SEQ ID NO: 132 - DNA, 111 bp, Homo sapiens
  source 1..111: mol_type = genomic DNA
aatatcatggctggattgcaacaaaccaacagtgaaaagattctcctgagctgggtctgacaatcaactcgtaattatccacaggttaatgtaatcaacttcaccaccagc

SEQ ID NO: 133 - DNA, 111 bp, Homo sapiens
  source 1..111: mol_type = genomic DNA
acaattggcatgcacttatcccaagcggtgaaagctggctgcccccttgatttggagtgagcaggcctgactccagaggttcagaagattattgctgatgttatccgaaac

SEQ ID NO: 134 - DNA, 111 bp, Homo sapiens
  source 1..111: mol_type = genomic DNA
gagaagtctgccgttactgccctgtggggcaaggtgaacgtggatgaagttggtggttaggccctgggcaggctgctggtggtctacccttggacccagaggttctttgag

SEQ ID NO: 135 - DNA, 111 bp, Homo sapiens
  source 1..111: mol_type = genomic DNA
gacctcaccccagacgaggtggtggccctagtgggccagggcctgcaggagggggagtgagacttcggggtcaaggcccggtccatcctgtgctgcatgcgccaccagccc

SEQ ID NO: 136 - DNA, 111 bp, Homo sapiens
  source 1..111: mol_type = genomic DNA
tttccttcccaggatcagatggcatctcctgaggttcccattgaagctggccagtattgatctaagagaaaacctcctcatgggggagaaagaaaggagaaggagcaccag

SEQ ID NO: 137 - DNA, 111 bp, Homo sapiens
  source 1..111: mol_type = genomic DNA
acctgcaggcaggcaacgctcaccttgacccagggtccatcttgctgggatgatgtttgaattccaaaccggatgagtggtgaatgccaatccccacactgccctgggact

SEQ ID NO: 138 - DNA, 111 bp, Homo sapiens
  source 1..111: mol_type = genomic DNA
tgggagattcctgatgggcagattacagtgggacaaagaattggatctggatcattttgaacagtctacaagggaaagtggcatggtgatgtggcagtgaaaatgttgaat

SEQ ID NO: 139 - DNA, 111 bp, Homo sapiens
  source 1..111: mol_type = genomic DNA
aaacaagtggttatagatggtgaaacctgtttgttggacatactggatacagctggataagaagagtacagtgccatgagagaccaatacatgaggacaggcgaaggcttc

SEQ ID NO: 140 - DNA, 35 bp, synthetic construct
  source 1..35: mol_type = other DNA
ggcgcctttggtgctcttcatcttgttggtcatgc

SEQ ID NO: 141 - DNA, 35 bp, synthetic construct; identical to SEQ ID NO: 126
  source 1..35: mol_type = other DNA

SEQ ID NO: 142 - DNA, 35 bp, synthetic construct
  source 1..35: mol_type = other DNA
gaagtggtagaagccgtagcccatcacgtggctca

SEQ ID NO: 143 - DNA, 35 bp, synthetic construct
  source 1..35: mol_type = other DNA
gaagtggtagaagccgtggcccatcacgtggctca

SEQ ID NO: 144 - DNA, 35 bp, synthetic construct
  source 1..35: mol_type = other DNA
cgtagccgctggggtaggtgccgaagtggtagaag

SEQ ID NO: 145 - DNA, 35 bp, synthetic construct
  source 1..35: mol_type = other DNA
gccgccgttgttgatggcgtgcaggaaggggttct

SEQ ID NO: 146 - DNA, 35 bp, synthetic construct
  source 1..35: mol_type = other DNA
gcatgaccaacaagatgaagagcaccaaaggcgcc

SEQ ID NO: 147 - DNA, 35 bp, synthetic construct
  source 1..35: mol_type = other DNA
tgagccacgtgatgggctacggcttctaccacttc

SEQ ID NO: 148 - DNA, 35 bp, synthetic construct
  source 1..35: mol_type = other DNA
tgagccacgtgatgggccacggcttctaccacttc

SEQ ID NO: 149 - DNA, 35 bp, synthetic construct
  source 1..35: mol_type = other DNA
cttctaccacttcggcacctaccccagcggctacg

SEQ ID NO: 150 - DNA, 35 bp, synthetic construct
  source 1..35: mol_type = other DNA
agaaccccttcctgcacgccatcaacaacggcggc

SEQ ID NO: 151 - DNA, 15 bp, synthetic construct
  source 1..15: mol_type = other DNA
gcaggaaggggttct

SEQ ID NO: 152 - DNA, 25 bp, synthetic construct
  source 1..25: mol_type = other DNA
ttgatggcgtgcaggaaggggttct

SEQ ID NO: 153 - DNA, 45 bp, synthetic construct
  source 1..45: mol_type = other DNA
tgttggtgtagccgccgttgttgatggcgtgcaggaaggggttct

SEQ ID NO: 154 - DNA, 55 bp, synthetic construct
  source 1..55: mol_type = other DNA
tcgatgcgggtgttggtgtagccgccgttgttgatggcgtgcaggaaggggttct

SEQ ID NO: 155 - DNA, 75 bp, synthetic construct
  source 1..75: mol_type = other DNA
cgccgccgtcctcgtacttctcgatgcgggtgttggtgtagccgccgttgttgatggcgtgcaggaaggggttct

SEQ ID NO: 156 - DNA, 79 bp, synthetic construct; identical to SEQ ID NO: 5
  source 1..79: mol_type = other DNA
  modified_base 41: mod_base = OTHER; note = 2'-O, 4'-C-methylene bridged nucleic acid

SEQ ID NO: 157 - DNA, 79 bp, synthetic construct; identical to SEQ ID NO: 5
  source 1..79: mol_type = other DNA
  modified_base 42: mod_base = OTHER; note = 2'-O, 4'-C-methylene bridged nucleic acid

SEQ ID NO: 158 - DNA, 79 bp, synthetic construct; identical to SEQ ID NO: 5
  source 1..79: mol_type = other DNA
  modified_base 43: mod_base = OTHER; note = 2'-O, 4'-C-methylene bridged nucleic acid

SEQ ID NO: 159 - DNA, 79 bp, synthetic construct; identical to SEQ ID NO: 5
  source 1..79: mol_type = other DNA
  modified_base 44: mod_base = OTHER; note = 2'-O, 4'-C-methylene bridged nucleic acid

SEQ ID NO: 160 - DNA, 79 bp, synthetic construct; identical to SEQ ID NO: 5
  source 1..79: mol_type = other DNA
  modified_base 45: mod_base = OTHER; note = 2'-O, 4'-C-methylene bridged nucleic acid

SEQ ID NO: 161 - DNA, 79 bp, synthetic construct; identical to SEQ ID NO: 5
  source 1..79: mol_type = other DNA
  modified_base 46: mod_base = OTHER; note = 2'-O, 4'-C-methylene bridged nucleic acid

SEQ ID NO: 162 - DNA, 79 bp, synthetic construct; identical to SEQ ID NO: 5
  source 1..79: mol_type = other DNA
  modified_base 39: mod_base = OTHER; note = 2'-O, 4'-C-methylene bridged nucleic acid

SEQ ID NO: 163 - DNA, 79 bp, synthetic construct; identical to SEQ ID NO: 5
  source 1..79: mol_type = other DNA
  modified_base 38: mod_base = OTHER; note = 2'-O, 4'-C-methylene bridged nucleic acid

SEQ ID NO: 164 - DNA, 79 bp, synthetic construct; identical to SEQ ID NO: 5
  source 1..79: mol_type = other DNA
  modified_base 37: mod_base = OTHER; note = 2'-O, 4'-C-methylene bridged nucleic acid

SEQ ID NO: 165 - DNA, 79 bp, synthetic construct; identical to SEQ ID NO: 5
  source 1..79: mol_type = other DNA
  modified_base 36: mod_base = OTHER; note = 2'-O, 4'-C-methylene bridged nucleic acid

SEQ ID NO: 166 - DNA, 79 bp, synthetic construct; identical to SEQ ID NO: 5
  source 1..79: mol_type = other DNA
  modified_base 35: mod_base = OTHER; note = 2'-O, 4'-C-methylene bridged nucleic acid

SEQ ID NO: 167 - DNA, 79 bp, synthetic construct; identical to SEQ ID NO: 5
  source 1..79: mol_type = other DNA
  modified_base 34: mod_base = OTHER; note = 2'-O, 4'-C-methylene bridged nucleic acid

SEQ ID NO: 168 - DNA, 79 bp, synthetic construct; identical to SEQ ID NO: 5
  source 1..79: mol_type = other DNA
  modified_base 38: mod_base = OTHER; note = 2'-O, 4'-C-methylene bridged nucleic acid
  modified_base 42: mod_base = OTHER; note = 2'-O, 4'-C-methylene bridged nucleic acid

SEQ ID NO: 169 - DNA, 79 bp, synthetic construct; identical to SEQ ID NO: 5
  source 1..79: mol_type = other DNA
  modified_base 37: mod_base = OTHER; note = 2'-O, 4'-C-methylene bridged nucleic acid
  modified_base 43: mod_base = OTHER; note = 2'-O, 4'-C-methylene bridged nucleic acid

SEQ ID NO: 170 - DNA, 79 bp, synthetic construct; identical to SEQ ID NO: 5
  source 1..79: mol_type = other DNA
  modified_base 36: mod_base = OTHER; note = 2'-O, 4'-C-methylene bridged nucleic acid
  modified_base 44: mod_base = OTHER; note = 2'-O, 4'-C-methylene bridged nucleic acid

SEQ ID NO: 171 - DNA, 79 bp, synthetic construct; identical to SEQ ID NO: 5
  source 1..79: mol_type = other DNA
  modified_base 35: mod_base = OTHER; note = 2'-O, 4'-C-methylene bridged nucleic acid
  modified_base 45: mod_base = OTHER; note = 2'-O, 4'-C-methylene bridged nucleic acid

SEQ ID NO: 172 - DNA, 79 bp, synthetic construct; identical to SEQ ID NO: 5
  source 1..79: mol_type = other DNA
  modified_base 34: mod_base = OTHER; note = 2'-O, 4'-C-methylene bridged nucleic acid
  modified_base 46: mod_base = OTHER; note = 2'-O, 4'-C-methylene bridged nucleic acid

SEQ ID NO: 173 - DNA, 79 bp, synthetic construct; identical to SEQ ID NO: 5
  source 1..79: mol_type = other DNA
  modified_base 35: mod_base = OTHER; note = 2'-O, 4'-C-methylene bridged nucleic acid
  modified_base 37: mod_base = OTHER; note = 2'-O, 4'-C-methylene bridged nucleic acid

SEQ ID NO: 174 - DNA, 79 bp, synthetic construct; identical to SEQ ID NO: 5
  source 1..79: mol_type = other DNA
  modified_base 36: mod_base = OTHER; note = 2'-O, 4'-C-methylene bridged nucleic acid
  modified_base 38: mod_base = OTHER; note = 2'-O, 4'-C-methylene bridged nucleic acid

SEQ ID NO: 175 - DNA, 79 bp, synthetic construct; identical to SEQ ID NO: 5
  source 1..79: mol_type = other DNA
  modified_base 37: mod_base = OTHER; note = 2'-O, 4'-C-methylene bridged nucleic acid
  modified_base 39: mod_base = OTHER; note = 2'-O, 4'-C-methylene bridged nucleic acid

SEQ ID NO: 176 - DNA, 79 bp, synthetic construct; identical to SEQ ID NO: 5
  source 1..79: mol_type = other DNA
  modified_base 41: mod_base = OTHER; note = 2'-O, 4'-C-methylene bridged nucleic acid
  modified_base 43: mod_base = OTHER; note = 2'-O, 4'-C-methylene bridged nucleic acid

SEQ ID NO: 177 - DNA, 79 bp, synthetic construct; identical to SEQ ID NO: 5
  source 1..79: mol_type = other DNA
  modified_base 42: mod_base = OTHER; note = 2'-O, 4'-C-methylene bridged nucleic acid
  modified_base 44: mod_base = OTHER; note = 2'-O, 4'-C-methylene bridged nucleic acid

SEQ ID NO: 178 - DNA, 79 bp, synthetic construct; identical to SEQ ID NO: 5
  source 1..79: mol_type = other DNA
  modified_base 43: mod_base = OTHER; note = 2'-O, 4'-C-methylene bridged nucleic acid
  modified_base 45: mod_base = OTHER; note = 2'-O, 4'-C-methylene bridged nucleic acid

SEQ ID NO: 179 - DNA, 79 bp, synthetic construct; identical to SEQ ID NO: 5
  source 1..79: mol_type = other DNA
  modified_base 40: mod_base = OTHER; note = 2'-O, 4'-C-methylene bridged nucleic acid
  modified_base 41: mod_base = OTHER; note = 2'-O, 4'-C-methylene bridged nucleic acid

SEQ ID NO: 180 - DNA, 79 bp, synthetic construct; identical to SEQ ID NO: 5
  source 1..79: mol_type = other DNA
  modified_base 40: mod_base = OTHER; note = 2'-O, 4'-C-methylene bridged nucleic acid
  modified_base 42: mod_base = OTHER; note = 2'-O, 4'-C-methylene bridged nucleic acid

SEQ ID NO: 181 - DNA, 79 bp, synthetic construct; identical to SEQ ID NO: 5
  source 1..79: mol_type = other DNA
  modified_base 40: mod_base = OTHER; note = 2'-O, 4'-C-methylene bridged nucleic acid
  modified_base 43: mod_base = OTHER; note = 2'-O, 4'-C-methylene bridged nucleic acid

SEQ ID NO: 182 - DNA, 79 bp, synthetic construct; identical to SEQ ID NO: 5
  source 1..79: mol_type = other DNA
  modified_base 40: mod_base = OTHER; note = 2'-O, 4'-C-methylene bridged nucleic acid
  modified_base 44: mod_base = OTHER; note = 2'-O, 4'-C-methylene bridged nucleic acid

SEQ ID NO: 183 - DNA, 79 bp, synthetic construct; identical to SEQ ID NO: 5
  source 1..79: mol_type = other DNA
  modified_base 40: mod_base = OTHER; note = 2'-O, 4'-C-methylene bridged nucleic acid
  modified_base 45: mod_base = OTHER; note = 2'-O, 4'-C-methylene bridged nucleic acid

SEQ ID NO: 184 - DNA, 79 bp, synthetic construct; identical to SEQ ID NO: 5
  source 1..79: mol_type = other DNA
  modified_base 40: mod_base = OTHER; note = 2'-O, 4'-C-methylene bridged nucleic acid
  modified_base 46: mod_base = OTHER; note = 2'-O, 4'-C-methylene bridged nucleic acid

SEQ ID NO: 185 - DNA, 79 bp, synthetic construct; identical to SEQ ID NO: 5
  source 1..79: mol_type = other DNA
  modified_base 40: mod_base = OTHER; note = 2'-O, 4'-C-methylene bridged nucleic acid
  modified_base 47: mod_base = OTHER; note = 2'-O, 4'-C-methylene bridged nucleic acid

SEQ ID NO: 186 - DNA, 79 bp, synthetic construct; identical to SEQ ID NO: 5
  source 1..79: mol_type = other DNA
  modified_base 39: mod_base = OTHER; note = 2'-O, 4'-C-methylene bridged nucleic acid
  modified_base 40: mod_base = OTHER; note = 2'-O, 4'-C-methylene bridged nucleic acid

SEQ ID NO: 187 - DNA, 79 bp, synthetic construct; identical to SEQ ID NO: 5
  source 1..79: mol_type = other DNA
  modified_base 38: mod_base = OTHER; note = 2'-O, 4'-C-methylene bridged nucleic acid
  modified_base 40: mod_base = OTHER; note = 2'-O, 4'-C-methylene bridged nucleic acid

SEQ ID NO: 188 - DNA, 79 bp, synthetic construct; identical to SEQ ID NO: 5
  source 1..79: mol_type = other DNA
  modified_base 37: mod_base = OTHER; note = 2'-O, 4'-C-methylene bridged nucleic acid
  modified_base 40: mod_base = OTHER; note = 2'-O, 4'-C-methylene bridged nucleic acid

SEQ ID NO: 189 - DNA, 79 bp, synthetic construct; identical to SEQ ID NO: 5
  source 1..79: mol_type = other DNA
  modified_base 36: mod_base = OTHER; note = 2'-O, 4'-C-methylene bridged nucleic acid
  modified_base 40: mod_base = OTHER; note = 2'-O, 4'-C-methylene bridged nucleic acid

SEQ ID NO: 190 - DNA, 79 bp, synthetic construct; identical to SEQ ID NO: 5
  source 1..79: mol_type = other DNA
  modified_base 35: mod_base = OTHER; note = 2'-O, 4'-C-methylene bridged nucleic acid
  modified_base 40: mod_base = OTHER; note = 2'-O, 4'-C-methylene bridged nucleic acid

SEQ ID NO: 191 - DNA, 79 bp, synthetic construct; identical to SEQ ID NO: 5
  source 1..79: mol_type = other DNA
  modified_base 34: mod_base = OTHER; note = 2'-O, 4'-C-methylene bridged nucleic acid
  modified_base 40: mod_base = OTHER; note = 2'-O, 4'-C-methylene bridged nucleic acid

SEQ ID NO: 192 - DNA, 79 bp, synthetic construct; identical to SEQ ID NO: 5
  source 1..79: mol_type = other DNA
  modified_base 33: mod_base = OTHER; note = 2'-O, 4'-C-methylene bridged nucleic acid
  modified_base 40: mod_base = OTHER; note = 2'-O, 4'-C-methylene bridged nucleic acid

SEQ ID NO: 193 - DNA, 79 bp, synthetic construct; identical to SEQ ID NO: 5
  source 1..79: mol_type = other DNA
  modified_base 40: mod_base = OTHER; note = 2'-O, 4'-C-methylene bridged nucleic acid
  modified_base 38: mod_base = OTHER; note = 2'-O, 4'-C-methylene bridged nucleic acid
  modified_base 42: mod_base = OTHER; note = 2'-O, 4'-C-methylene bridged nucleic acid

SEQ ID NO: 194 - DNA, 79 bp, synthetic construct; identical to SEQ ID NO: 5
  source 1..79: mol_type = other DNA
  modified_base 40: mod_base = OTHER; note = 2'-O, 4'-C-methylene bridged nucleic acid
  modified_base 37: mod_base = OTHER; note = 2'-O, 4'-C-methylene bridged nucleic acid
  modified_base 43: mod_base = OTHER; note = 2'-O, 4'-C-methylene bridged nucleic acid

SEQ ID NO: 195 - DNA, 79 bp, synthetic construct; identical to SEQ ID NO: 5
  source 1..79: mol_type = other DNA
  modified_base 40: mod_base = OTHER; note = 2'-O, 4'-C-methylene bridged nucleic acid
  modified_base 36: mod_base = OTHER; note = 2'-O, 4'-C-methylene bridged nucleic acid
  modified_base 44: mod_base = OTHER; note = 2'-O, 4'-C-methylene bridged nucleic acid

SEQ ID NO: 196 - DNA, 79 bp, synthetic construct; identical to SEQ ID NO: 5
  source 1..79: mol_type = other DNA
  modified_base 40: mod_base = OTHER; note = 2'-O, 4'-C-methylene bridged nucleic acid
  modified_base 35: mod_base = OTHER; note = 2'-O, 4'-C-methylene bridged nucleic acid
  modified_base 45: mod_base = OTHER; note = 2'-O, 4'-C-methylene bridged nucleic acid

SEQ ID NO: 197 - DNA, 79 bp, synthetic construct; identical to SEQ ID NO: 5
  source 1..79: mol_type = other DNA
  modified_base 40: mod_base = OTHER; note = 2'-O, 4'-C-methylene bridged nucleic acid
  modified_base 34: mod_base = OTHER; note = 2'-O, 4'-C-methylene bridged nucleic acid
  modified_base 46: mod_base = OTHER; note = 2'-O, 4'-C-methylene bridged nucleic acid

SEQ ID NO: 198 - DNA, 79 bp, synthetic construct; identical to SEQ ID NO: 5
  source 1..79: mol_type = other DNA
  modified_base 40: mod_base = OTHER; note = 2'-O, 4'-C-methylene bridged nucleic acid
  modified_base 33: mod_base = OTHER; note = 2'-O, 4'-C-methylene bridged nucleic acid
  modified_base 47: mod_base = OTHER; note = 2'-O, 4'-C-methylene bridged nucleic acid

SEQ ID NO: 199 - DNA, 79 bp, synthetic construct; identical to SEQ ID NO: 5
  source 1..79: mol_type = other DNA
  modified_base 38: mod_base = OTHER; note = 2'-O, 4'-C-methylene bridged nucleic acid
  modified_base 39: mod_base = OTHER; note = 2'-O, 4'-C-methylene bridged nucleic acid
  modified_base 41: mod_base = OTHER; note = 2'-O, 4'-C-methylene bridged nucleic acid
  modified_base 42: mod_base = OTHER; note = 2'-O, 4'-C-methylene bridged nucleic acid

SEQ ID NO: 200 - DNA, 79 bp, synthetic construct; identical to SEQ ID NO: 5
  source 1..79: mol_type = other DNA
  modified_base 37: mod_base = OTHER; note = 2'-O, 4'-C-methylene bridged nucleic acid
  modified_base 38: mod_base = OTHER; note = 2'-O, 4'-C-methylene bridged nucleic acid
  modified_base 42: mod_base = OTHER; note = 2'-O, 4'-C-methylene bridged nucleic acid
  modified_base 43: mod_base = OTHER; note = 2'-O, 4'-C-methylene bridged nucleic acid

SEQ ID NO: 201 - DNA, 79 bp, synthetic construct; identical to SEQ ID NO: 5
  source 1..79: mol_type = other DNA
  modified_base 37: mod_base = OTHER; note = 2'-O, 4'-C-methylene bridged nucleic acid
  modified_base 38: mod_base = OTHER; note = 2'-O, 4'-C-methylene bridged nucleic acid
  modified_base 39: mod_base = OTHER; note = 2'-O, 4'-C-methylene bridged nucleic acid
  modified_base 41: mod_base = OTHER; note = 2'-O, 4'-C-methylene bridged nucleic acid
  modified_base 42: mod_base = OTHER; note = 2'-O, 4'-C-methylene bridged nucleic acid
  modified_base 43: mod_base = OTHER; note = 2'-O, 4'-C-methylene bridged nucleic acid

SEQ ID NO: 202 - DNA, 79 bp, synthetic construct; identical to SEQ ID NO: 5
  source 1..79: mol_type = other DNA
  modified_base 39: mod_base = OTHER; note = 2'-O, 4'-C-methylene bridged nucleic acid
  modified_base 41: mod_base = OTHER; note = 2'-O, 4'-C-methylene bridged nucleic acid
  modified_base 44: mod_base = OTHER; note = 2'-O, 4'-C-methylene bridged nucleic acid

SEQ ID NO: 203 - DNA, 79 bp, synthetic construct; identical to SEQ ID NO: 5
  source 1..79: mol_type = other DNA
  modified_base 37: mod_base = OTHER; note = 2'-O, 4'-C-methylene bridged nucleic acid
  modified_base 39: mod_base = OTHER; note = 2'-O, 4'-C-methylene bridged nucleic acid
  modified_base 41: mod_base = OTHER; note = 2'-O, 4'-C-methylene bridged nucleic acid
  modified_base 43: mod_base = OTHER; note = 2'-O, 4'-C-methylene bridged nucleic acid
  modified_base 44: mod_base = OTHER; note = 2'-O, 4'-C-methylene bridged nucleic acid

SEQ ID NO: 204 - DNA, 79 bp, synthetic construct; identical to SEQ ID NO: 5
  source 1..79: mol_type = other DNA
  modified_base 40: mod_base = OTHER; note = 2'-O, 4'-C-methylene bridged nucleic acid
  modified_base 41: mod_base = OTHER; note = 2'-O, 4'-C-methylene bridged nucleic acid
  modified_base 44: mod_base = OTHER; note = 2'-O, 4'-C-methylene bridged nucleic acid

SEQ ID NO: 205 - DNA, 79 bp, synthetic construct; identical to SEQ ID NO: 5
  source 1..79: mol_type = other DNA
  modified_base 39: mod_base = OTHER; note = 2'-O, 4'-C-methylene bridged nucleic acid
  modified_base 40: mod_base = OTHER; note = 2'-O, 4'-C-methylene bridged nucleic acid
  modified_base 44: mod_base = OTHER; note = 2'-O, 4'-C-methylene bridged nucleic acid

SEQ ID NO: 206 - DNA, 79 bp, synthetic construct; identical to SEQ ID NO: 5
  source 1..79: mol_type = other DNA
  modified_base 40: mod_base = OTHER; note = 2'-O, 4'-C-methylene bridged nucleic acid
  modified_base 42: mod_base = OTHER; note = 2'-O, 4'-C-methylene bridged nucleic acid
  modified_base 44: mod_base = OTHER; note = 2'-O, 4'-C-methylene bridged nucleic acid

SEQ ID NO: 207 - DNA, 79 bp, synthetic construct; identical to SEQ ID NO: 5
  source 1..79: mol_type = other DNA
  modified_base 38: mod_base = OTHER; note = 2'-O, 4'-C-methylene bridged nucleic acid
  modified_base 40: mod_base = OTHER; note = 2'-O, 4'-C-methylene bridged nucleic acid
  modified_base 44: mod_base = OTHER; note = 2'-O, 4'-C-methylene bridged nucleic acid

SEQ ID NO: 208 - DNA, 34 bp, synthetic construct
  source 1..34: mol_type = other DNA
ctgaccttcagcccctacctgctgagccacgtga

SEQ ID NO: 209 - DNA, 33 bp, synthetic construct
  source 1..33: mol_type = other DNA
ctgaccttcagcccctacctgctgagccacgtg

SEQ ID NO: 210 - DNA, 32 bp, synthetic construct
  source 1..32: mol_type = other DNA
ctgaccttcagcccctacctgctgagccacgt

SEQ ID NO: 211 - DNA, 31 bp, synthetic construct
  source 1..31: mol_type = other DNA
ctgaccttcagcccctacctgctgagccacg

SEQ ID NO: 212 - DNA, 79 bp, synthetic construct
  source 1..79: mol_type = other DNA
tgattacattaacctgtggataattacgagttgattgtcggacccagctcaggagaatcttttcactgttggtttgttg

SEQ ID NO: 213 - DNA, 35 bp, synthetic construct
  source 1..35: mol_type = other DNA
caacaaaccaacagtgaaaagattctcctgagctg

SEQ ID NO: 214 - DNA, 65 bp, synthetic construct
  source 1..65: mol_type = other DNA
gccgggattctcctccacgtcaccgcatgttagaagacttcctctgccctcgctggtggtgaagt

SEQ ID NO: 215 - DNA, 79 bp, synthetic construct; identical to SEQ ID NO: 212
  source 1..79: mol_type = other DNA
  modified_base 40: mod_base = OTHER; note = 2'-O, 4'-C-methylene bridged nucleic acid
  modified_base 44: mod_base = OTHER; note = 2'-O, 4'-C-methylene bridged nucleic acid

SEQ ID NO: 216 - DNA, 79 bp, synthetic construct; identical to SEQ ID NO: 212
  source 1..79: mol_type = other DNA
  modified_base 36: mod_base = OTHER; note = 2'-O, 4'-C-methylene bridged nucleic acid
  modified_base 40: mod_base = OTHER; note = 2'-O, 4'-C-methylene bridged nucleic acid

SEQ ID NO: 217 - DNA, 79 bp, synthetic construct; identical to SEQ ID NO: 212
  source 1..79: mol_type = other DNA
  modified_base 39: mod_base = OTHER; note = 2'-O, 4'-C-methylene bridged nucleic acid
  modified_base 41: mod_base = OTHER; note = 2'-O, 4'-C-methylene bridged nucleic acid

SEQ ID NO: 218 - DNA, 79 bp, synthetic construct; identical to SEQ ID NO: 212
  source 1..79: mol_type = other DNA
  modified_base 40: mod_base = OTHER; note = 2'-O, 4'-C-methylene bridged nucleic acid

SEQ ID NO: 219 - DNA, 79 bp, synthetic construct; identical to SEQ ID NO: 212
  source 1..79: mol_type = other DNA
  modified_base 38: mod_base = OTHER; note = 2'-O, 4'-C-methylene bridged nucleic acid
  modified_base 42: mod_base = OTHER; note = 2'-O, 4'-C-methylene bridged nucleic acid

SEQ ID NO: 220 - DNA, 79 bp, synthetic construct
  source 1..79: mol_type = other DNA
cagcaataatcttctgaacctctggagtcaggcctgctcgctccaaatcaagggggcagccagctttcaccgcttggga

SEQ ID NO: 221 - DNA, 35 bp, synthetic construct
  source 1..35: mol_type = other DNA
tcccaagcggtgaaagctggctgcccccttgattt

SEQ ID NO: 222 - DNA, 65 bp, synthetic construct
  source 1..65: mol_type = other DNA
gccgggattctcctccacgtcaccgcatgttagaagacttcctctgccctcgtttcggataacat

SEQ ID NO: 223 - DNA, 79 bp, synthetic construct; identical to SEQ ID NO: 220
  source 1..79: mol_type = other DNA
  modified_base 40: mod_base = OTHER; note = 2'-O, 4'-C-methylene bridged nucleic acid
  modified_base 44: mod_base = OTHER; note = 2'-O, 4'-C-methylene bridged nucleic acid

SEQ ID NO: 224 - DNA, 79 bp, synthetic construct; identical to SEQ ID NO: 220
  source 1..79: mol_type = other DNA
  modified_base 36: mod_base = OTHER; note = 2'-O, 4'-C-methylene bridged nucleic acid
  modified_base 40: mod_base = OTHER; note = 2'-O, 4'-C-methylene bridged nucleic acid

SEQ ID NO: 225 - DNA, 79 bp, synthetic construct; identical to SEQ ID NO: 220
  source 1..79: mol_type = other DNA
  modified_base 39: mod_base = OTHER; note = 2'-O, 4'-C-methylene bridged nucleic acid
  modified_base 41: mod_base = OTHER; note = 2'-O, 4'-C-methylene bridged nucleic acid

SEQ ID NO: 226 - DNA, 79 bp, synthetic construct; identical to SEQ ID NO: 220
  source 1..79: mol_type = other DNA
  modified_base 40: mod_base = OTHER; note = 2'-O, 4'-C-methylene bridged nucleic acid

SEQ ID NO: 227 - DNA, 79 bp, synthetic construct; identical to SEQ ID NO: 220
  source 1..79: mol_type = other DNA
  modified_base 38: mod_base = OTHER; note = 2'-O, 4'-C-methylene bridged nucleic acid
  modified_base 42: mod_base = OTHER; note = 2'-O, 4'-C-methylene bridged nucleic acid

SEQ ID NO: 228 - DNA, 21 bp, synthetic construct
  source 1..21: mol_type = other DNA
gagcagactctaaatctgccg

SEQ ID NO: 229 - DNA, 21 bp, synthetic construct
  source 1..21: mol_type = other DNA
  modified_base 9^10: mod_base = OTHER; note = POCH2CH3 modification
gagcagactctaaatctgccg

SEQ ID NO: 230 - DNA, 21 bp, synthetic construct
  source 1..21: mol_type = other DNA
  modified_base 9^10: mod_base = OTHER; note = phosphorothioate bond
gagcagactctaaatctgccg

SEQ ID NO: 231 - DNA, 21 bp, synthetic construct
  source 1..21: mol_type = other DNA
  modified_base 10: mod_base = OTHER; note = 2'-O, 4'-C-methylene bridged nucleic acid
  modified_base 12: mod_base = OTHER; note = 2'-O, 4'-C-methylene bridged nucleic acid
gagcagactctaaatctgccg

SEQ ID NO: 232 - DNA, 21 bp, synthetic construct
  source 1..21: mol_type = other DNA
  modified_base 10: mod_base = OTHER; note = 2'-O, 4'-C-methylene bridged nucleic acid
  modified_base 12: mod_base = OTHER; note = 2'-O, 4'-C-methylene bridged nucleic acid
gagcagactccaaatctgccg